European Patent Specification EP 4 479 556 B1, published March 4, 2026. Title: INTERNAL CONTROLS FOR NUCLEIC ACID AMPLIFICATION. Applicant: Becton, Dickinson and Company. The sequence listing filed with the application follows.

SEQUENCE LISTING (6 sequences)

SEQ ID NO: 1 - protein, 775 aa, synthetic construct
MILDTDYITENGKPVIRVFKKENGEFKIEYDRTFEPYFYALLKDDSAIEDVKKVTAKRHGTVVKVKRAEKVQKKFLGRPIEVWKLYFNHPQDVPAIRDRIRAHPAVVDIYEYDIPFAKRYLIDKGLIPMEGDEELTMLAFDIETLYHEGEEFGTGPILMISYADGSEARVITWKKIDLPYVDVVSTEKEMIKRFLRVVREKDPDVLITYNGDNFDFAYLKKRCEELGIKFTLGRDGSEPKIQRMGDRFAVEVKGRIHFDLYPVIRRTINLPTYTLEAVYEAVFGKPKEKVYAEEIAQAWESGEGLERVARYSMEDAKVTYELGREFFPMEAQLSRLIGQSLWDVSRSSTGNLVEWFLLRKAYKRNELAPNKPDERELARRRGGYAGGYVKEPERGLWDNIVYLDFRSLYPSIIITHNVSPDTLNREGCKEYDVAPEVGHKFCKDFPGFIPSLLGDLLEERQKIKRKMKATVDPLEKKLLDYRQRAIKILANSFYGYYGYAKARWYCKECAESVTAWGREYIEMVIRELEEKFGFKVLYADTDGLHATIPGADAETVKKKAKEFLKYINPKLPGLLELEYEGFYVRGFFVTKKKYAVIDEEGKITTRGLEIVRRDWSEIAKETQARVLEAILKHGDVEEAVRIVKEVTEKLSKYEVPPEKLVIHEQITRDLRDYKATGPHVAVAKRLAARGVKIRPGTVISYIVLKGSGRIGDRAIPADEFDPTKHRYDAEYYIENQVLPAVERILKAFGYRKEDLRYQKTKQVGLGAWLKVKGKK

SEQ ID NO: 2 - protein, 775 aa, synthetic construct
MILDTDYITENGKPVIRVFKKENGEFKIEYDRTFEPYFYALLKDDSAIEDVKKVTAKRHGTVVKVKRAEKVQKKFLGRPIEVWKLYFNHPQDVPAIRDRIRAHPAVVDIYEYDIPFAKRYLIDKGLIPMEGDEELTMLAFDIDTLYHEGEEFGTGPILMISYADGSEARVITWKKIDLPYVDVVSTEKEMIKRFLRVVREKDPDVLITYNGDNFDFAYLKKRCEELGIKFTLGRDGSEPKIQRMGDRFAVEVKGRIHFDLYPVIRRTINLPTYTLEAVYEAVFGKPKEKVYAEEIAQAWESGEGLERVARYSMEDAKVTYELGREFFPMEAQLSRLIGQSLWDVSRSSTGNLVEWFLLRKAYKRNELAPNKPDERELARRRGGYAGGYVKEPERGLWDNIVYLDFRSLYPSIIITHNVSPDTLNREGCKEYDVAPEVGHKFCKDFPGFIPSLLGDLLEERQKIKRKMKATVDPLEKKLLDYRQRAIKILANSFYGYYGYAKARWYCKECAESVTAWGREYIEMVIRELEEKFGFKVLYADTDGLHATIPGADAETVKKKAKEFLKYINPKLPGLLELEYEGFYVRGFFVTKKKYAVIDEEGKITTRGLEIVRRDWSEIAKETQARVLEAILKHGDVEEAVRIVKEVTEKLSKYEVPPEKLVIHEQITRDLRDYKATGPHVAVAKRLAARGVKIRPGTVISYIVLKGSGRIGDRAIPADEFDPTKHRYDAEYYIENQVLPAVERILKAFGYRKEDLRYQKTKQVGLGAWLKVKGKK

SEQ ID NO: 3 - DNA, 13 bp, synthetic construct
  source 1..13: mol_type = other DNA
tgcgtgaaactcg

SEQ ID NO: 4 - DNA, 11 bp, synthetic construct
  source 1..11: mol_type = other DNA
ggaaatacgag

SEQ ID NO: 5 - DNA, 12 bp, synthetic construct
  source 1..12: mol_type = other DNA
ggaaatacgagt

SEQ ID NO: 6 - DNA, 14 bp, synthetic construct
  source 1..14: mol_type = other DNA
tgcgtgaatactcg